European Patent Application EP 4 215 203 A1, published July 26, 2023. Title: 一种用于冬季防治呼吸道疾病的药物组合物. Applicant: 天津中医药大学. The sequence listing filed with the application follows.

SEQUENCE LISTING (12 sequences)

SEQ ID NO: 1 - DNA, 22 bp, Artificial Sequence
  引物
ggtgagaagagatgtctgaatc

SEQ ID NO: 2 - DNA, 20 bp, Artificial Sequence
  引物
gtagggaagtgatgggagag

SEQ ID NO: 3 - DNA, 20 bp, Artificial Sequence
  引物
ggcactggcagaaaacaacc

SEQ ID NO: 4 - DNA, 21 bp, Artificial Sequence
  引物
gcaagtctcctcattgaatcc

SEQ ID NO: 5 - DNA, 23 bp, Artificial Sequence
  引物
gcacctccactccatcctgaagg

SEQ ID NO: 6 - DNA, 24 bp, Artificial Sequence
  引物
ccattacagggctcctgagcattg

SEQ ID NO: 7 - DNA, 20 bp, Artificial Sequence
  引物
ccagggacaggtatggagca

SEQ ID NO: 8 - DNA, 23 bp, Artificial Sequence
  引物
ttcaacacgcaggacaggtacag

SEQ ID NO: 9 - DNA, 18 bp, Artificial Sequence
  引物
gcggtgcttgttcctcag

SEQ ID NO: 10 - DNA, 19 bp, Artificial Sequence
  引物
ggctacaggcttgtcactc

SEQ ID NO: 11 - DNA, 20 bp, Artificial Sequence
  引物
atgattctacccacggcaag

SEQ ID NO: 12 - DNA, 20 bp, Artificial Sequence
  引物
ctggaagatggtgatgggtt